European Patent Application EP 4 491 628 A1, published January 15, 2025. Title: Production method for Fc-containing molecular modification reagent. Applicant: 日本メジフィジックス株式会社. Application JP. The sequence listing filed with the application follows.

SEQUENCE LISTING (134 sequences)

SEQ ID NO: 1 - protein, 13 aa, synthetic construct
  SITE 6: note = X is K, C, D, E, R, V, F, L, 2-Aminooctanedioic acid, Dpr, Orn, AcOrn, AcDab, Dab, Nle, Nva, Tle, Ala(t-Bu), or Cha
  REGION 1..13: note = Fc binding peptide
DCAYHXGELVWCT

SEQ ID NO: 2 - protein, 17 aa, synthetic construct
  REGION 1..17: note = IgG binding peptide
  SITE 8: note = X is K,C,D,E,R,V, F, L, 2-Aminooctanedioic acid, Dpr, Orn, AcOrn, AcDab, Dab, Nle, Nva, Tle, Ala(t-Bu), or Cha
GPDCAYHXGELVWCTFH

SEQ ID NO: 3 - protein, 13 aa, synthetic construct
  REGION 1..13: note = IgG binding peptide
  SITE 6: note = X is K,C,D,E,R,V, F, L, 2-Aminooctanedioic acid, Dpr, Orn, AcOrn, AcDab, Dab, Nle, Nva, Tle, Ala(t-Bu), or Cha
RCAYHXGELVWCS

SEQ ID NO: 4 - protein, 17 aa, synthetic construct
  REGION 1..17: note = IgG binding peptide
  SITE 8: note = X is K,C,D,E,R,V, F, L, 2-Aminooctanedioic acid, Dpr, Orn, AcOrn, AcDab, Dab, Nle, Nva, Tle, Ala(t-Bu), or Cha
GPRCAYHXGELVWCSFH

SEQ ID NO: 5 - protein, 17 aa, synthetic construct
  REGION 1..17: note = IgG binding peptide
  SITE 8: note = X is K,C,D,E,R,V, F, L, 2-Aminooctanedioic acid, Dpr, Orn, AcOrn, AcDab, Dab, Nle, Nva, Tle, Ala(t-Bu), or Cha
SPDCAYHXGELVWCTFH

SEQ ID NO: 6 - protein, 17 aa, synthetic construct
  REGION 1..17: note = IgG binding peptide
  SITE 8: note = X is K,C,D,E,R,V, F, L, 2-Aminooctanedioic acid, Dpr, Orn, AcOrn, AcDab, Dab, Nle, Nva, Tle, Ala(t-Bu), or Cha
GDDCAYHXGELVWCTFH

SEQ ID NO: 7 - protein, 17 aa, synthetic construct
  REGION 1..17: note = IgG binding peptide
  SITE 8: note = X is K,C,D,E,R,V, F, L, 2-Aminooctanedioic acid, Dpr, Orn, AcOrn, AcDab, Dab, Nle, Nva, Tle, Ala(t-Bu), or Cha
GPSCAYHXGELVWCTFH

SEQ ID NO: 8 - protein, 17 aa, synthetic construct
  REGION 1..17: note = IgG binding peptide
  SITE 8: note = X is K,C,D,E,R,V, F, L, 2-Aminooctanedioic acid, Dpr, Orn, AcOrn, AcDab, Dab, Nle, Nva, Tle, Ala(t-Bu), or Cha
GPDCAYHXGELVWCSFH

SEQ ID NO: 9 - protein, 17 aa, synthetic construct
  REGION 1..17: note = IgG binding peptide
  SITE 8: note = X is K,C,D,E,R,V, F, L, 2-Aminooctanedioic acid, Dpr, Orn, AcOrn, AcDab, Dab, Nle, Nva, Tle, Ala(t-Bu), or Cha
GPDCAYHXGELVWCTHH

SEQ ID NO: 10 - protein, 17 aa, synthetic construct
  REGION 1..17: note = IgG binding peptide
  SITE 8: note = X is K,C,D,E,R,V, F, L, 2-Aminooctanedioic acid, Dpr, Orn, AcOrn, AcDab, Dab, Nle, Nva, Tle, Ala(t-Bu), or Cha
GPDCAYHXGELVWCTFY

SEQ ID NO: 11 - protein, 17 aa, synthetic construct
  REGION 1..17: note = IgG binding peptide
  SITE 8: note = X is K,C,D,E,R,V, F, L, 2-Aminooctanedioic acid, Dpr, Orn, AcOrn, AcDab, Dab, Nle, Nva, Tle, Ala(t-Bu), or Cha
SPDCAYHXGELVWCTFY

SEQ ID NO: 12 - protein, 17 aa, synthetic construct
  REGION 1..17: note = IgG binding peptide
  SITE 8: note = X is K,C,D,E,R,V, F, L, 2-Aminooctanedioic acid, Dpr, Orn, AcOrn, AcDab, Dab, Nle, Nva, Tle, Ala(t-Bu), or Cha
SDDCAYHXGELVWCTFY

SEQ ID NO: 13 - protein, 17 aa, synthetic construct
  REGION 1..17: note = IgG binding peptide
  SITE 8: note = X is K,C,D,E,R,V, F, L, 2-Aminooctanedioic acid, Dpr, Orn, AcOrn, AcDab, Dab, Nle, Nva, Tle, Ala(t-Bu), or Cha
RGNCAYHXGQLVWCTYH

SEQ ID NO: 14 - protein, 17 aa, synthetic construct
  REGION 1..17: note = IgG binding peptide
  SITE 2: note = X is homocysteine
  SITE 8: note = X is K,C,D,E,R,V, F, L, 2-Aminooctanedioic acid, Dpr, Orn, AcOrn, AcDab, Dab, Nle, Nva, Tle, Ala(t-Bu), or Cha
  SITE 16: note = X is homocysteine
GXDCAYHXGELVWCTXH

SEQ ID NO: 15 - protein, 19 aa, synthetic construct
  REGION 1..19: note = IgG binding peptide
  SITE 10: note = X is K,C,D,E,R,V, F, L, 2-Aminooctanedioic acid, Dpr, Orn, AcOrn, AcDab, Dab, Nle, Nva, Tle, Ala(t-Bu), or Cha
RRGPDCAYHXGELVWCTFH

SEQ ID NO: 16 - protein, 13 aa, synthetic construct
  REGION 1..13: note = IgG binding peptide
  SITE 6: note = X is K,C,D,E,R,V, F, L, 2-Aminooctanedioic acid, Dpr, Orn, AcOrn, AcDab, Dab, Nle, Nva, Tle, Ala(t-Bu), or Cha
DCTYHXGNLVWCT

SEQ ID NO: 17 - protein, 13 aa, synthetic construct
  REGION 1..13: note = IgG binding peptide
  SITE 6: note = X is K,C,D,E,R,V, F, L, 2-Aminooctanedioic acid, Dpr, Orn, AcOrn, AcDab, Dab, Nle, Nva, Tle, Ala(t-Bu), or Cha
DCAYHXGNLVWCT

SEQ ID NO: 18 - protein, 13 aa, synthetic construct
  REGION 1..13: note = IgG binding peptide
  SITE 6: note = X is K,C,D,E,R,V, F, L, 2-Aminooctanedioic acid, Dpr, Orn, AcOrn, AcDab, Dab, Nle, Nva, Tle, Ala(t-Bu), or Cha
DCTYHXGELVWCT

SEQ ID NO: 19 - protein, 13 aa, synthetic construct
  REGION 1..13: note = IgG binding peptide
  SITE 6: note = X is K,C,D,E,R,V, F, L, 2-Aminooctanedioic acid, Dpr, Orn, AcOrn, AcDab, Dab, Nle, Nva, Tle, Ala(t-Bu), or Cha
DCAWHXGELVWCT

SEQ ID NO: 20 - protein, 13 aa, synthetic construct
  REGION 1..13: note = IgG binding peptide
  SITE 6: note = X is K,C,D,E,R,V, F, L, 2-Aminooctanedioic acid, Dpr, Orn, AcOrn, AcDab, Dab, Nle, Nva, Tle, Ala(t-Bu), or Cha
DCTYTXGNLVWCT

SEQ ID NO: 21 - protein, 13 aa, synthetic construct
  REGION 1..13: note = IgG binding peptide
  SITE 6: note = X is K,C,D,E,R,V, F, L, 2-Aminooctanedioic acid, Dpr, Orn, AcOrn, AcDab, Dab, Nle, Nva, Tle, Ala(t-Bu), or Cha
DCAYTXGNLVWCT

SEQ ID NO: 22 - protein, 13 aa, synthetic construct
  REGION 1..13: note = IgG binding peptide
  SITE 6: note = X is K,C,D,E,R,V, F, L, 2-Aminooctanedioic acid, Dpr, Orn, AcOrn, AcDab, Dab, Nle, Nva, Tle, Ala(t-Bu), or Cha
DCSYTXGNLVWCT

SEQ ID NO: 23 - protein, 13 aa, synthetic construct
  REGION 1..13: note = IgG binding peptide
  SITE 6: note = X is K,C,D,E,R,V, F, L, 2-Aminooctanedioic acid, Dpr, Orn, AcOrn, AcDab, Dab, Nle, Nva, Tle, Ala(t-Bu), or Cha
DCTWTXGNLVWCT

SEQ ID NO: 24 - protein, 13 aa, synthetic construct
  REGION 1..13: note = IgG binding peptide
  SITE 6: note = X is K,C,D,E,R,V, F, L, 2-Aminooctanedioic acid, Dpr, Orn, AcOrn, AcDab, Dab, Nle, Nva, Tle, Ala(t-Bu), or Cha
DCTYHXGNLVWCT

SEQ ID NO: 25 - protein, 13 aa, synthetic construct
  REGION 1..13: note = IgG binding peptide
  SITE 6: note = X is K,C,D,E,R,V, F, L, 2-Aminooctanedioic acid, Dpr, Orn, AcOrn, AcDab, Dab, Nle, Nva, Tle, Ala(t-Bu), or Cha
DCTYRXGNLVWCT

SEQ ID NO: 26 - protein, 13 aa, synthetic construct
  REGION 1..13: note = IgG binding peptide
  SITE 6: note = X is K,C,D,E,R,V, F, L, 2-Aminooctanedioic acid, Dpr, Orn, AcOrn, AcDab, Dab, Nle, Nva, Tle, Ala(t-Bu), or Cha
DCTYSXGNLVWCT

SEQ ID NO: 27 - protein, 13 aa, synthetic construct
  REGION 1..13: note = IgG binding peptide
  SITE 6: note = X is K,C,D,E,R,V, F, L, 2-Aminooctanedioic acid, Dpr, Orn, AcOrn, AcDab, Dab, Nle, Nva, Tle, Ala(t-Bu), or Cha
DCTYTXGNLVWCT

SEQ ID NO: 28 - protein, 13 aa, synthetic construct
  REGION 1..13: note = IgG binding peptide
  SITE 6: note = X is K,C,D,E,R,V, F, L, 2-Aminooctanedioic acid, Dpr, Orn, AcOrn, AcDab, Dab, Nle, Nva, Tle, Ala(t-Bu), or Cha
DCTYTXGELVWCT

SEQ ID NO: 29 - protein, 13 aa, synthetic construct
  REGION 1..13: note = IgG binding peptide
  SITE 6: note = X is K,C,D,E,R,V, F, L, 2-Aminooctanedioic acid, Dpr, Orn, AcOrn, AcDab, Dab, Nle, Nva, Tle, Ala(t-Bu), or Cha
DCTYTXGRLVWCT

SEQ ID NO: 30 - protein, 13 aa, synthetic construct
  REGION 1..13: note = IgG binding peptide
  SITE 6: note = X is K,C,D,E,R,V, F, L, 2-Aminooctanedioic acid, Dpr, Orn, AcOrn, AcDab, Dab, Nle, Nva, Tle, Ala(t-Bu), or Cha
DCTYTXGDLVWCT

SEQ ID NO: 31 - protein, 13 aa, synthetic construct
  REGION 1..13: note = IgG binding peptide
  SITE 6: note = X is K,C,D,E,R,V, F, L, 2-Aminooctanedioic acid, Dpr, Orn, AcOrn, AcDab, Dab, Nle, Nva, Tle, Ala(t-Bu), or Cha
DCTYTXGNLIWCT

SEQ ID NO: 32 - protein, 13 aa, synthetic construct
  REGION 1..13: note = IgG binding peptide
DCAYHRGELVWCT

SEQ ID NO: 33 - protein, 17 aa, synthetic construct
  REGION 1..17: note = IgG binding peptide
GPDCAYHRGELVWCTFH

SEQ ID NO: 34 - protein, 13 aa, synthetic construct
  REGION 1..13: note = IgG binding peptide
RCAYHRGELVWCS

SEQ ID NO: 35 - protein, 17 aa, synthetic construct
  REGION 1..17: note = IgG binding peptide
GPRCAYHRGELVWCSFH

SEQ ID NO: 36 - protein, 17 aa, synthetic construct
  REGION 1..17: note = IgG binding peptide
SPDCAYHRGELVWCTFH

SEQ ID NO: 37 - protein, 17 aa, synthetic construct
  REGION 1..17: note = IgG binding peptide
GDDCAYHRGELVWCTFH

SEQ ID NO: 38 - protein, 17 aa, synthetic construct
  REGION 1..17: note = IgG binding peptide
GPSCAYHRGELVWCTFH

SEQ ID NO: 39 - protein, 17 aa, synthetic construct
  REGION 1..17: note = IgG binding peptide
GPDCAYHRGELVWCSFH

SEQ ID NO: 40 - protein, 17 aa, synthetic construct
  REGION 1..17: note = IgG binding peptide
GPDCAYHRGELVWCTHH

SEQ ID NO: 41 - protein, 17 aa, synthetic construct
  REGION 1..17: note = IgG binding peptide
GPDCAYHRGELVWCTFY

SEQ ID NO: 42 - protein, 17 aa, synthetic construct
  REGION 1..17: note = IgG binding peptide
SPDCAYHRGELVWCTFY

SEQ ID NO: 43 - protein, 17 aa, synthetic construct
  REGION 1..17: note = IgG binding peptide
SDDCAYHRGELVWCTFY

SEQ ID NO: 44 - protein, 13 aa, synthetic construct
  REGION 1..13: note = IgG binding peptide
DCTYHRGNLVWCT

SEQ ID NO: 45 - protein, 13 aa, synthetic construct
  REGION 1..13: note = IgG binding peptide
DCAYHRGNLVWCT

SEQ ID NO: 46 - protein, 13 aa, synthetic construct
  REGION 1..13: note = IgG binding peptide
DCTYHRGELVWCT

SEQ ID NO: 47 - protein, 13 aa, synthetic construct
  REGION 1..13: note = IgG binding peptide
DCAWHRGELVWCT

SEQ ID NO: 48 - protein, 13 aa, synthetic construct
  REGION 1..13: note = IgG binding peptide
DCTYTNGNLVWCT

SEQ ID NO: 49 - protein, 13 aa, synthetic construct
  REGION 1..13: note = IgG binding peptide
DCAYTNGNLVWCT

SEQ ID NO: 50 - protein, 13 aa, synthetic construct
  REGION 1..13: note = IgG binding peptide
DCSYTNGNLVWCT

SEQ ID NO: 51 - protein, 13 aa, synthetic construct
  REGION 1..13: note = IgG binding peptide
DCTWTNGNLVWCT

SEQ ID NO: 52 - protein, 13 aa, synthetic construct
  REGION 1..13: note = IgG binding peptide
DCTYHNGNLVWCT

SEQ ID NO: 53 - protein, 13 aa, synthetic construct
  REGION 1..13: note = IgG binding peptide
DCTYRNGNLVWCT

SEQ ID NO: 54 - protein, 13 aa, synthetic construct
  REGION 1..13: note = IgG binding peptide
DCTYSNGNLVWCT

SEQ ID NO: 55 - protein, 13 aa, synthetic construct
  REGION 1..13: note = IgG binding peptide
DCTYTRGNLVWCT

SEQ ID NO: 56 - protein, 13 aa, synthetic construct
  REGION 1..13: note = IgG binding peptide
DCTYTNGELVWCT

SEQ ID NO: 57 - protein, 13 aa, synthetic construct
  REGION 1..13: note = IgG binding peptide
DCTYTNGRLVWCT

SEQ ID NO: 58 - protein, 13 aa, synthetic construct
  REGION 1..13: note = IgG binding peptide
DCTYTNGDLVWCT

SEQ ID NO: 59 - protein, 13 aa, synthetic construct
  REGION 1..13: note = IgG binding peptide
DCTYTNGNLIWCT

SEQ ID NO: 60 - protein, 22 aa, synthetic construct
  REGION 1..22: note = IgG binding peptide
GSGGSGPDCAYHRGELVWCTFH

SEQ ID NO: 61 - protein, 18 aa, synthetic construct
  REGION 1..18: note = IgG binding peptide
GSGGSDCAYHRGELVWCT

SEQ ID NO: 62 - protein, 23 aa, synthetic construct
  REGION 1..23: note = IgG binding peptide
KRRRGSGPDCAYHKGELVWCTFH

SEQ ID NO: 63 - protein, 23 aa, synthetic construct
  REGION 1..23: note = IgG binding peptide
KEEGGSGPDCAYHKGELVWCTFH

SEQ ID NO: 64 - protein, 17 aa, synthetic construct
  REGION 1..17: note = IgG binding peptide
GPDCAYHKGELVWCTFH

SEQ ID NO: 65 - protein, 22 aa, synthetic construct
  REGION 1..22: note = IgG binding peptide
RRRGSGPDCAYHKGELVWCTFH

SEQ ID NO: 66 - protein, 22 aa, synthetic construct
  REGION 1..22: note = IgG binding peptide
EEGGSGPDCAYHKGELVWCTFH

SEQ ID NO: 67 - protein, 19 aa, synthetic construct
  REGION 1..19: note = IgG binding peptide
KRRRGSDCAYHKGELVWCT

SEQ ID NO: 68 - protein, 19 aa, synthetic construct
  REGION 1..19: note = IgG binding peptide
KEEGGSDCAYHKGELVWCT

SEQ ID NO: 69 - protein, 13 aa, synthetic construct
  REGION 1..13: note = IgG binding peptide
DCAYHKGELVWCT

SEQ ID NO: 70 - protein, 18 aa, synthetic construct
  REGION 1..18: note = IgG binding peptide
RRRGSDCAYHKGELVWCT

SEQ ID NO: 71 - protein, 18 aa, synthetic construct
  REGION 1..18: note = IgG binding peptide
EEGGSDCAYHKGELVWCT

SEQ ID NO: 72 - protein, 34 aa, synthetic construct
  REGION 1..34: note = IgG binding peptide
FNMQCQRRFYEALHDPNLNEEQRNARIRSIRDDC

SEQ ID NO: 73 - protein, 35 aa, synthetic construct
  REGION 1..35: note = IgG binding peptide
GFNMQCQRRFYEALHDPNLNEEQRNARIRSIRDDC

SEQ ID NO: 74 - protein, 34 aa, synthetic construct
  REGION 1..34: note = IgG binding peptide
KNMQCQRRFYEALHDPNLNEEQRNARIRSIRDDC

SEQ ID NO: 75 - protein, 35 aa, synthetic construct
  REGION 1..35: note = IgG binding peptide
GFNMQCQKRFYEALHDPNLNEEQRNARIRSIRDDC

SEQ ID NO: 76 - protein, 34 aa, synthetic construct
  REGION 1..34: note = IgG binding peptide
KNMQCQKRFYEALHDPNLNEEQRNARIRSIRDDC

SEQ ID NO: 77 - protein, 33 aa, synthetic construct
  REGION 1..33: note = IgG binding peptide
FNMQQQRRFYEALHDPNLNEEQRNARIRSIRDD

SEQ ID NO: 78 - protein, 35 aa, synthetic construct
  REGION 1..35: note = IgG binding peptide
GKNMQCQRRFYEALHDPNLNEEQRNARIRSIRDDC

SEQ ID NO: 79 - protein, 40 aa, synthetic construct
  REGION 1..40: note = IgG binding peptide
FNMQQQRRFYEALHDPNLNEEQRNARIRSIRDDPSGSGSK

SEQ ID NO: 80 - protein, 40 aa, synthetic construct
  REGION 1..40: note = IgG binding peptide
FNMQCQRRFYEALHDPNLNEEQRNARIRSIRDDCSGSGSK

SEQ ID NO: 81 - protein, 34 aa, synthetic construct
  REGION 1..34: note = IgG binding peptide
FNMQQQRRFYEALHDPNLNEEQRNARIRSIRDDP

SEQ ID NO: 82 - protein, 33 aa, synthetic construct
  REGION 1..33: note = IgG binding peptide
FNMQQQCRFYEALHDPNLNEEQRNARIRSIRDD

SEQ ID NO: 83 - protein, 34 aa, synthetic construct
  REGION 1..34: note = IgG binding peptide
FNMQQQRRFYEALHDPNLNEEQRNARIRSIRDDC

SEQ ID NO: 84 - protein, 39 aa, synthetic construct
  REGION 1..39: note = IgG binding peptide
FNMQQQRRFYEALHDPNLNEEQRNARIRSIRDDPSRRKR

SEQ ID NO: 85 - protein, 39 aa, synthetic construct
  REGION 1..39: note = IgG binding peptide
FNMQQQRRFYEALHDPNLNEEQRNARIRSIRDDPSRRCR

SEQ ID NO: 86 - protein, 44 aa, synthetic construct
  REGION 1..44: note = IgG binding peptide
FNMQQQCRFYEALHDPNLNEEQRNARICSIRDDPSRRCRRCRRC

SEQ ID NO: 87 - protein, 44 aa, synthetic construct
  REGION 1..44: note = IgG binding peptide
FNMQQQKRFYEALHDPNLNEEQRNARIKSIRDDPSRRKRRKRRK

SEQ ID NO: 88 - protein, 33 aa, synthetic construct
  REGION 1..33: note = IgG binding peptide
KNMQQQCRFYEALHDPNLNEEQRNARIRSIRDD

SEQ ID NO: 89 - protein, 34 aa, synthetic construct
  REGION 1..34: note = IgG binding peptide
KNMQQQRRFYEALHDPNLNEEQRNARIRSIRDDC

SEQ ID NO: 90 - protein, 39 aa, synthetic construct
  REGION 1..39: note = IgG binding peptide
KNMQQQRRFYEALHDPNLNEEQRNARIRSIRDDPSRRKR

SEQ ID NO: 91 - protein, 39 aa, synthetic construct
  REGION 1..39: note = IgG binding peptide
KNMQQQRRFYEALHDPNLNEEQRNARIRSIRDDPSRRCR

SEQ ID NO: 92 - protein, 44 aa, synthetic construct
  REGION 1..44: note = IgG binding peptide
KNMQQQCRFYEALHDPNLNEEQRNARICSIRDDPSRRCRRCRRC

SEQ ID NO: 93 - protein, 44 aa, synthetic construct
  REGION 1..44: note = IgG binding peptide
KNMQQQKRFYEALHDPNLNEEQRNARIKSIRDDPSRRKRRKRRK

SEQ ID NO: 94 - protein, 34 aa, synthetic construct
  REGION 1..34: note = IgG binding peptide
GFNMQQQCRFYEALHDPNLNEEQRNARIRSIRDD

SEQ ID NO: 95 - protein, 35 aa, synthetic construct
  REGION 1..35: note = IgG binding peptide
GFNMQQQRRFYEALHDPNLNEEQRNARIRSIRDDC

SEQ ID NO: 96 - protein, 40 aa, synthetic construct
  REGION 1..40: note = IgG binding peptide
GFNMQQQRRFYEALHDPNLNEEQRNARIRSIRDDPSRRKR

SEQ ID NO: 97 - protein, 40 aa, synthetic construct
  REGION 1..40: note = IgG binding peptide
GFNMQQQRRFYEALHDPNLNEEQRNARIRSIRDDPSRRCR

SEQ ID NO: 98 - protein, 45 aa, synthetic construct
  REGION 1..45: note = IgG binding peptide
GFNMQQQCRFYEALHDPNLNEEQRNARICSIRDDPSRRCRRCRRC

SEQ ID NO: 99 - protein, 45 aa, synthetic construct
  REGION 1..45: note = IgG binding peptide
GFNMQQQKRFYEALHDPNLNEEQRNARIKSIRDDPSRRKRRKRRK

SEQ ID NO: 100 - protein, 34 aa, synthetic construct
  REGION 1..34: note = IgG binding peptide
FNMQCQZRFYEALHDPNLNEEQRNARIRSIRDDC

SEQ ID NO: 101 - protein, 34 aa, synthetic construct
  REGION 1..34: note = IgG binding peptide
KNMQCQZRFYEALHDPNLNEEQRNARIRSIRDDC

SEQ ID NO: 102 - protein, 40 aa, synthetic construct
  REGION 1..40: note = IgG binding peptide
GFNMQCQKRFYEALHDPNLNEEQRNARIRSIRDDCSRRKR

SEQ ID NO: 103 - protein, 34 aa, synthetic construct
  REGION 1..34: note = IgG binding peptide
FNMQCQKRFYEALHDPNLNEEQRNARIRSIRDDC

SEQ ID NO: 104 - protein, 39 aa, synthetic construct
  REGION 1..39: note = IgG binding peptide
KNMQCQKRFYEALHDPNLNEEQRNARIRSIRDDCSRRKR

SEQ ID NO: 105 - protein, 45 aa, synthetic construct
  REGION 1..45: note = IgG binding peptide
GFNMQCQKRFYEALHDPNLNEEQRNARIRSIRDDCSRRKRRKRRK

SEQ ID NO: 106 - protein, 44 aa, synthetic construct
  REGION 1..44: note = IgG binding peptide
KNMQCQKRFYEALHDPNLNEEQRNARIRSIRDDCSRRKRRKRRK

SEQ ID NO: 107 - protein, 45 aa, synthetic construct; identical to SEQ ID NO: 105
  REGION 1..45: note = IgG binding peptide

SEQ ID NO: 108 - protein, 11 aa, synthetic construct
  REGION 1..11: note = IgG binding peptide
CAWHLGELVWC

SEQ ID NO: 109 - protein, 13 aa, synthetic construct
  REGION 1..13: note = IgG binding peptide
DCAWHLGELVWCT

SEQ ID NO: 110 - protein, 13 aa, synthetic construct
  REGION 1..13: note = IgG binding peptide
DCAWHLGELVFCT

SEQ ID NO: 111 - protein, 13 aa, synthetic construct
  REGION 1..13: note = IgG binding peptide
  SITE 11: note = X is 1-naphtoyl, 2-naphtoyl, benzyl, or benzothiophene
DCAWHLGELVXCT

SEQ ID NO: 112 - protein, 15 aa, synthetic construct
  REGION 1..15: note = IgG binding peptide
CDCAWHLGELVWCTC

SEQ ID NO: 113 - protein, 11 aa, synthetic construct
  REGION 1..11: note = IgG binding peptide
CAYHLGELVWC

SEQ ID NO: 114 - protein, 14 aa, synthetic construct
  REGION 1..14: note = IgG binding peptide
DCAYHLGELVWCTF

SEQ ID NO: 115 - protein, 23 aa, synthetic construct
  REGION 1..23: note = IgG binding peptide
KRRRGSGPDCAYHKGELVWCTFH

SEQ ID NO: 116 - protein, 13 aa, synthetic construct
  REGION 1..13: note = Peptide for modifying antibody
DCAYHKGELVWCT

SEQ ID NO: 117 - protein, 17 aa, synthetic construct
  REGION 1..17: note = Peptide for modifying antibody
GPDCAYHKGELVWCTFH

SEQ ID NO: 118 - protein, 13 aa, synthetic construct
  REGION 1..13: note = Peptide for modifying antibody
RCAYHKGELVWCS

SEQ ID NO: 119 - protein, 17 aa, synthetic construct
  REGION 1..17: note = Peptide for modifying antibody
GPRCAYHKGELVWCSFH

SEQ ID NO: 120 - protein, 17 aa, synthetic construct
  REGION 1..17: note = Peptide for modifying antibody
SPDCAYHKGELVWCTFH

SEQ ID NO: 121 - protein, 17 aa, synthetic construct
  REGION 1..17: note = Peptide for modifying antibody
GDDCAYHKGELVWCTFH

SEQ ID NO: 122 - protein, 17 aa, synthetic construct
  REGION 1..17: note = Peptide for modifying antibody
GPSCAYHKGELVWCTFH

SEQ ID NO: 123 - protein, 17 aa, synthetic construct
  REGION 1..17: note = Peptide for modifying antibody
GPDCAYHKGELVWCSFH

SEQ ID NO: 124 - protein, 17 aa, synthetic construct
  REGION 1..17: note = Peptide for modifying antibody
GPDCAYHKGELVWCTHH

SEQ ID NO: 125 - protein, 17 aa, synthetic construct
  REGION 1..17: note = Peptide for modifying antibody
GPDCAYHKGELVWCTFY

SEQ ID NO: 126 - protein, 17 aa, synthetic construct
  REGION 1..17: note = Peptide for modifying antibody
SPDCAYHKGELVWCTFY

SEQ ID NO: 127 - protein, 17 aa, synthetic construct
  REGION 1..17: note = Peptide for modifying antibody
SDDCAYHKGELVWCTFY

SEQ ID NO: 128 - protein, 17 aa, synthetic construct
  REGION 1..17: note = Peptide for modifying antibody
RGNCAYHKGQLVWCTYH

SEQ ID NO: 129 - protein, 17 aa, synthetic construct
  REGION 1..17: note = Peptide for modifying antibody
  SITE 2: note = X is a homosysteine residue.
  SITE 16: note = X is a homosysteine residue.
GXDCAYHKGELVWCTXH

SEQ ID NO: 130 - protein, 13 aa, synthetic construct
  REGION 1..13: note = Peptide for modifying antibody
DCTYHKGNLVWCT

SEQ ID NO: 131 - protein, 13 aa, synthetic construct
  REGION 1..13: note = Peptide for modifying antibody
DCAYHKGNLVWCT

SEQ ID NO: 132 - protein, 13 aa, synthetic construct
  REGION 1..13: note = Peptide for modifying antibody
DCTYHKGELVWCT

SEQ ID NO: 133 - protein, 13 aa, synthetic construct
  REGION 1..13: note = Peptide for modifying antibody
DCAWHKGELVWCT

SEQ ID NO: 134 - protein, 17 aa, synthetic construct
  REGION 1..17: note = Peptide for modifying antibody
  DISULFID 4..14: note = interchain cross-link
GPDCAYHKGELVWCTFH